European Patent Specification EP 3 773 686 B1, published June 7, 2023. Title: ALKALINE PHOSPHATASE AGENTS FOR TREATMENT OF RADIATION DISORDERS. Applicant: Synthetic Biologics, Inc. Kaleko, Michael Furlan Freguia, Christian Connelly, Sheila. The sequence listing filed with the application follows.

SEQUENCE LISTING (60 sequences)

SEQ ID NO: 1 - protein, 528 aa, Artificial Sequence
  Synthetic polymer
MQGPWVLLLLGLRLQLSLGVIPAEEENPAFWNRQAAEALDAAKKLQPIQKVAKNLILFLGDGLGVPTVTATRILKGQKNGKLGPETPLAMDRFPYLALSKTYNVDRQVPDSAATATAYLCGVKANFQTIGLSAAARFNQCNTTRGNEVISVMNRAKQAGKSVGVVTTTRVQHASPAGTYAHTVNRNWYSDADMPASARQEGCQDIATQLISNMDIDVILGGGRKYMFPMGTPDPEYPADASQNGIRLDGKNLVQEWLAKHQGAWYVWNRTELMQASLDQSVTHLMGLFEPGDTKYEIHRDPTLDPSLMEMTEAALRLLSRNPRGFYLFVEGGRIDHGHHEGVAYQALTEAVMFDDAIERAGQLTSEEDTLTLVTADHSHVFSFGGYTLRGSSIFGLAPSKAQDSKAYTSILYGNGPGYVFNSGVRPDVNESESGSPDYQQQAAVPLSSETHGGEDVAVFARGPQAHLVHGVQEQSFVAHVMAFAACLEPYTACDLAPPACTTDAAHPVAASLPLLAGTLLLLGASAAP

SEQ ID NO: 2 - protein, 533 aa, Artificial Sequence
  Synthetic polymer
MQGACVLLLLGLHLQLSLGLIPAEEENPAFWNRQAAQALDVAKKLQPIQTAAKNVILFLGDGMGVPTVTATRILKGQMNGKLGPETPLAMDQFPYVALSKTYNVDRQVPDSAGTATAYLCGVKGNYRTIGVSAAARYNQCNTTRGNEVTSVINRAKKAGKAVGVVTTTRVQHASPAGAYAHTVNRNWYSDADLPADAQKNGCQDIAAQLVYNMDIDVILGGGRMYMFPEGTPDPEYPDDASVNGVRKDKQNLVQEWQAKHQGAQYVWNRTALLQAADDSSVTHLMGLFEPADMKYNVQQDHTKDPTLAEMTEAALQVLSRNPRGFYLFVEGGRIDHGHHDGKAYMALTEAIMFDNAIAKANELTSELDTLILVTADHSHVFSFGGYTLRGTSIFGLAPGKALDSKSYTSILYGNGPGYALGGGSRPDVNGSTSEEPSYRQQAAVPLASETHGGEDVAVFARGPQAHLVHGVQEETFVAHIMAFAGCVEPYTDCNLPAPATATSIPDAAHLAASPPPLALLAGAMLLLLAPTLY

SEQ ID NO: 3 - protein, 530 aa, Artificial Sequence
  Synthetic polymer
MQWACVLLLLGLWLQLSLTFIPAEEEDPAFWNRQAAQALDVAKKLQPIQTAAKNVILFLGDGMGVPTVTATRILKGQMNGKLGPETPLAMDQFPYVALSKTYNVDRQVPDSAGTATAYLCGVKGNYKTIGVSAAARYNQCNTTSGNEVTSVMNRAKKAGKSVGVVTTSRVQHASPAGAYAHTVNRNWYSDADLPADAQTYGCQDIATQLVNNMDIDVILGGGRMYMFPEGTPDPEYPYDVNQTGVRKDKRNLVQEWQAKHQGAQYVWNRTELLQAANDPSVTHLMGLFEPADMKYNVQQDPTKDPTLEEMTEAALQVLSRNPQGFYLFVEGGRIDHGHHEGKAYMALTDTVMFDNAIAKANELTSELDTLILATADHSHVFSFGGYTLRGTSIFGLAPSKASDNKSYTSILYGNGPGYVLGGGLRPDVNDSISEDPSYRQQAAVPLSSESHGGEDVAVFARGPQAHLVHGVQEETFVAHVMAFAGCVEPYTDCNLPAPSGLSDAAHLAASPPSLALLAGAMLLLLAPALY

SEQ ID NO: 4 - protein, 503 aa, Artificial Sequence
  Synthetic polymer
MQGPWVLLLLGLRLQLSLGVIPAEEENPAFWNRQAAEALDAAKKLQPIQKVAKNLILFLGDGLGVPTVTATRILKGQKNGKLGPETPLAMDRFPYLALSKTYNVDRQVPDSAATATAYLCGVKANFQTIGLSAAARFNQCNTTRGNEVISVMNRAKQAGKSVGVVTTTRVQHASPAGTYAHTVNRNWYSDADMPASARQEGCQDIATQLISNMDIDVILGGGRKYMFPMGTPDPEYPADASQNGIRLDGKNLVQEWLAKHQGAWYVWNRTELMQASLDQSVTHLMGLFEPGDTKYEIHRDPTLDPSLMEMTEAALRLLSRNPRGFYLFVEGGRIDHGHHEGVAYQALTEAVMFDDAIERAGQLTSEEDTLTLVTADHSHVFSFGGYTLRGSSIFGLAPSKAQDSKAYTSILYGNGPGYVFNSGVRPDVNESESGSPDYQQQAAVPLSSETHGGEDVAVFARGPQAHLVHGVQEQSFVAHVMAFAACLEPYTACDLAPPAGTTD

SEQ ID NO: 5 - protein, 506 aa, Artificial Sequence
  Synthetic polymer
MQGACVLLLLGLHLQLSLGLIPAEEENPAFWNRQAAQALDVAKKLQPIQTAAKNVILFLGDGMGVPTVTATRILKGQMNGKLGPETPLAMDQFPYVALSKTYNVDRQVPDSAGTATAYLCGVKGNYRTIGVSAAARYNQCNTTRGNEVTSVINRAKKAGKAVGVVTTTRVQHASPAGAYAHTVNRNWYSDADLPADAQKNGCQDIAAQLVYNMDIDVILGGGRMYMFPEGTPDPEYPDDASVNGVRKDKQNLVQEWQAKHQGAQYVWNRTALLQAADDSSVTHLMGLFEPADMKYNVQQDHTKDPTLAEMTEAALQVLSRNPRGFYLFVEGGRIDHGHHDGKAYMALTEAIMFDNAIAKANELTSELDTLILVTADHSHVFSFGGYTLRGTSIFGLAPGKALDSKSYTSILYGNGPGYALGGGSRPDVNGSTSEEPSYRQQAAVPLASETHGGEDVAVFARGPQAHLVHGVQEETFVAHIMAFAGCVEPYTDCNLPAPATATSIPD

SEQ ID NO: 6 - protein, 503 aa, Artificial Sequence
  Synthetic polymer
MQWACVLLLLGLWLQLSLTFIPAEEEDPAFWNRQAAQALDVAKKLQPIQTAAKNVILFLGDGMGVPTVTATRILKGQMNGKLGPETPLAMDQFPYVALSKTYNVDRQVPDSAGTATAYLCGVKGNYKTIGVSAAARYNQCNTTSGNEVTSVMNRAKKAGKSVGVVTTSRVQHASPAGAYAHTVNRNWYSDADLPADAQTYGCQDIATQLVNNMDIDVILGGGRMYMFPEGTPDPEYPYDVNQTGVRKDKRNLVQEWQAKHQGAQYVWNRTELLQAANDPSVTHLMGLFEPADMKYNVQQDPTKDPTLEEMTEAALQVLSRNPQGFYLFVEGGRIDHGHHEGKAYMALTDTVMFDNAIAKANELTSELDTLILATADHSHVFSFGGYTLRGTSIFGLAPSKASDNKSYTSILYGNGPGYVLGGGLRPDVNDSISEDPSYRQQAAVPLSSESHGGEDVAVFARGPQAHLVHGVQEETFVAHVMAFAGCVEPYTDCNLPAPSGLSD

SEQ ID NO: 7 - protein, 508 aa, Artificial Sequence
  Synthetic polymer
MQWACVLLLLGLWLQLSLTFIPAEEEDPAFWNRQAAQALDVAKKLQPIQTAAKNVILFLGDGMGVPTVTATRILKGQMNGKLGPETPLAMDQFPYVALSKTYNVDRQVPDSAGTATAYLCGVKGNYKTIGVSAAARYNQCNTTSGNEVTSVMNRAKKAGKSVGVVTTSRVQHASPAGAYAHTVNRNWYSDADLPADAQTYGCQDIATQLVNNMDIDVILGGGRMYMFPEGTPDPEYPYDVNQTGVRKDKRNLVQEWQAKHQGAQYVWNRTELLQAANDPSVTHLMGLFEPADMKYNVQQDPTKDPTLEEMTEAALQVLSRNPQGFYLFVEGGRIDHGHHEGKAYMALTDTVMFDNAIAKANELTSELDTLILATADHSHVFSFGGYTLRGTSIFGLAPSKASDNKSYTSILYGNGPGYVLGGGLRPDVNDSISEDPSYRQQAAVPLSSESHGGEDVAVFARGPQAHLVHGVQEETFVAHVMAFAGCVEPYTDCNLPAPSGLSDAAHLA

SEQ ID NO: 8 - protein, 754 aa, Artificial Sequence
  Synthetic polymer
MQGACVLLLLGLHLQLSLGLIPAEEENPAFWNRQAAQALDVAKKLQPIQTAAKNVILFLGDGMGVPTVTATRILKGQMNGKLGPETPLAMDQFPYVALSKTYNVDRQVPDSAGTATAYLCGVKGNYRTIGVSAAARYNQCNTTRGNEVTSVINRAKKAGKAVGVVTTTRVQHASPAGAYAHTVNRNWYSDADLPADAQKNGCQDIAAQLVYNMDIDVILGGGRMYMFPEGTPDPEYPDDASVNGVRKDKQNLVQEWQAKHQGAQYVWNRTALLQAADDSSVTHLMGLFEPADMKYNVQQDHTKDPTLAEMTEAALQVLSRNPRGFYLFVEGGRIDHGHHDGKAYMALTEAIMFDNAIAKANELTSELDTLILVTADHSHVFSFGGYTLRGTSIFGLAPGKALDSKSYTSILYGNGPGYALGGGSRPDVNGSTSEEPSYRQQAAVPLASETHGGEDVAVFARGPQAHLVHGVQEETFVAHIMAFAGCVEPYTDCNLPAPATATSIPDGGSGGSGGGGSGGGGSEPKSCDKTHTCPPCPAPELLGGPSVFLFPPKPKDTLMISRTPEVTCVVVDVSHEDPQVKFNWYVDGVQVHNAKTKPREQQYNSTYRVVSVLTVLHQNWLDGKEYKCKVSNKALPAPIEKTISKAKGQPREPQVYTLPPSREEMTKNQVSLTCLVKGFYPSDIAVEWESNGQPENNYKTTPPVLDSDGSFFLYSKLTVDKSRWQQGNVFSCSVMHEALHNHYTQKSLSLSPGK

SEQ ID NO: 9 - protein, 751 aa, Artificial Sequence
  Synthetic polymer
MQWACVLLLLGLWLQLSLTFIPAEEEDPAFWNRQAAQALDVAKKLQPIQTAAKNVILFLGDGMGVPTVTATRILKGQMNGKLGPETPLAMDQFPYVALSKTYNVDRQVPDSAGTATAYLCGVKGNYKTIGVSAAARYNQCNTTSGNEVTSVMNRAKKAGKSVGVVTTSRVQHASPAGAYAHTVNRNWYSDADLPADAQTYGCQDIATQLVNNMDIDVILGGGRMYMFPEGTPDPEYPYDVNQTGVRKDKRNLVQEWQAKHQGAQYVWNRTELLQAANDPSVTHLMGLFEPADMKYNVQQDPTKDPTLEEMTEAALQVLSRNPQGFYLFVEGGRIDHGHHEGKAYMALTDTVMFDNAIAKANELTSELDTLILATADHSHVFSFGGYTLRGTSIFGLAPSKASDNKSYTSILYGNGPGYVLGGGLRPDVNDSISEDPSYRQQAAVPLSSESHGGEDVAVFARGPQAHLVHGVQEETFVAHVMAFAGCVEPYTDCNLPAPSGLSDGGSGGSGGGGSGGGGSEPKSCDKTHTCPPCPAPELLGGPSVFLFPPKPKDTLMISRTPEVTCVVVDVSHEDPQVKFNWYVDGVQVHNAKTKPREQQYNSTYRVVSVLTVLHQNWLDGKEYKCKVSNKALPAPIEKTISKAKGQPREPQVYTLPPSREEMTKNQVSLTCLVKGFYPSDIAVEWESNGQPENNYKTTPPVLDSDGSFFLYSKLTVDKSRWQQGNVFSCSVMHEALHNHYTQKSLSLSPGK

SEQ ID NO: 10 - protein, 539 aa, Artificial Sequence
  Synthetic polymer
MQWACVLLLLGLWLQLSLTFIPAEEEDPAFWNRQAAQALDVAKKLQPIQTAAKNVILFLGDGMGVPTVTATRILKGQMNGKLGPETPLAMDQFPYVALSKTYNVDRQVPDSAGTATAYLCGVKGNYKTIGVSAAARYNQCNTTSGNEVTSVMNRAKKAGKSVGVVTTSRVQHASPAGAYAHTVNRNWYSDADLPADAQTYGCQDIATQLVNNMDIDVILGGGRMYMFPEGTPDPEYPYDVNQTGVRKDKRNLVQEWQAKHQGAQYVWNRTELLQAANDPSVTHLMGLFEPADMKYNVQQDPTKDPTLEEMTEAALQVLSRNPQGFYLFVEGGRIDHGHHEGKAYMALTDTVMFDNAIAKANELTSELDTLILATADHSHVFSFGGYTLRGTSIFGLAPSKASDNKSYTSILYGNGPGYVLGGGLRPDVNDSISEDPSYRQQAAVPLSSESHGGEDVAVFARGPQAHLVHGVQEETFVAHVMAFAGCVEPYTDCNLEVLFQGPAPPAGTTDAAHPGRSVVPALLPLRAGTLLLLETATAP

SEQ ID NO: 11 - protein, 534 aa, Artificial Sequence
  Synthetic polymer
MQWACVLLLLGLWLQLSLTFIPAEEEDPAFWNRQAAQALDVAKKLQPIQTAAKNVILFLGDGMGVPTVTATRILKGQMNGKLGPETPLAMDQFPYVALSKTYNVDRQVPDSAGTATAYLCGVKGNYKTIGVSAAARYNQCNTTSGNEVTSVMNRAKKAGKSVGVVTTSRVQHASPAGAYAHTVNRNWYSDADLPADAQTYGCQDIATQLVNNMDIDVILGGGRMYMFPEGTPDPEYPYDVNQTGVRKDKRNLVQEWQAKHQGAQYVWNRTELLQAANDPSVTHLMGLFEPADMKYNVQQDPTKDPTLEEMTEAALQVLSRNPQGFYLFVEGGRIDHGHHEGKAYMALTDTVMFDNAIAKANELTSELDTLILATADHSHVFSFGGYTLRGTSIFGLAPSKASDNKSYTSILYGNGPGYVLGGGLRPDVNDSISEDPSYRQQAAVPLSSESHGGEDVAVFARGPQAHLVHGVQEETFVAHVMAFAGCVEPYTDCNLAPPAGTTDAAHPIEGRSVVPALLPLRAGTLLLLETATAP

SEQ ID NO: 12 - DNA, 1669 bp, Artificial Sequence
  Synthetic polymer
atgcaggggccctgggtgctgctgctgctgggcctgaggctacagctctccctgggcgtcatcccaggtaatgaggctccccaagctgttccacacacagggcaccccctcagccaggctgacctgatctctactctccccctggccagctgaggaggagaacccggccttctggaaccgccaggcagctgaggccctggatgctgccaagaagctgcagcccatccagaaggtcgccaagaacctcatcctcttcctgggcgatgggttgggggtgcccacggtgacagccaccaggatcctaaaggggcagaagaatggcaaactggggcctgagacgcccctggccatggaccgcttcccatacctggctctgtccaagacatacaatgtggacagacaggtgccagacagcgcagccacagccacggcctacctgtgcggggtcaaggccaacttccagaccatcggcttgagtgcagccgcccgctttaaccagtgcaacacgacacgcggcaatgaggtcatctccgtgatgaaccgggccaagcaagcaggaaagtcagtaggagtggtgaccaccacacgggtgcagcacgcctcgccagccggcacctacgcacacacagtgaaccgcaactggtactcagatgctgacatgcctgcctcagcccgccaggaggggtgccaggacatcgccactcagctcatctccaacatggacattgacgtgatccttggcggaggccgcaagtacatgtttcccatggggaccccagaccctgagtacccagctgatgccagccagaatggaatcaggctggacgggaagaacctggtgcaggaatggctggcaaagcaccagggtgcctggtatgtgtggaaccgcactgagctcatgcaggcgtccctggaccagtctgtgacccatctcatgggcctctttgagcccggagacacgaaatatgagatccaccgagaccccacactggacccctccctgatggagatgacagaggctgccctgcgcctgctgagcaggaacccccgcggcttctacctctttgtggagggcggccgcatcgaccatggtcatcatgagggtgtggcttaccaggcactcactgaggcggtcatgttcgacgacgccattgagagggcgggccagctcaccagcgaggaggacacgctgaccctcgtcaccgctgaccactcccatgtcttctcctttggtggctacaccttgcgagggagctccatcttcgggttggcccccagcaaggctcaggacagcaaagcctacacgtccatcctgtacggcaatggcccgggctacgtgttcaactcaggcgtgcgaccagacgtgaatgagagcgagagcgggagccccgattaccagcagcaggcggcggtgcccctgtcgtccgagacccacggaggcgaagacgtggcggtgtttgcgcgcggcccgcaggcgcacctggtgcatggtgtgcaggagcagagcttcgtagcgcatgtcatggccttcgctgcctgtctggagccctacacggcctgcgacctggcgcctcccgcctgcaccaccgacgccgcgcacccagttgccgcgtcgctgccactgctggccgggaccctgctgctgctgggggcgtccgctgctccctga

SEQ ID NO: 13 - DNA, 1671 bp, Artificial Sequence
  Synthetic polymer
atgcaggggccctgggtgctgctgctgctgggcctgaggctacagctctccctgggcgtcatcccagctgaggaggagaacccggccttctggaaccgccaggcagctgaggccctggatgctgccaagaagctgcagcccatccagaaggtcgccaagaacctcatcctcttcctgggcgatgggttgggggtgcccacggtgacagccaccaggatcctaaaggggcagaagaatggcaaactggggcctgagacgcccctggccatggaccgcttcccatacctggctctgtccaagacatacaatgtggacagacaggtgccagacagcgcagccacagccacggcctacctgtgcggggtcaaggccaacttccagaccatcggcttgagtgcagccgcccgctttaaccagtgcaacacgacacgcggcaatgaggtcatctccgtgatgaaccgggccaagcaagcaggaaagtcagtaggagtggtgaccaccacacgggtgcagcacgcctcgccagccggcacctacgcacacacagtgaaccgcaactggtactcagatgctgacatgcctgcctcagcccgccaggaggggtgccaggacatcgccactcagctcatctccaacatggacattgacgtgatccttggcggaggccgcaagtacatgtttcccatggggaccccagaccctgagtacccagctgatgccagccagaatggaatcaggctggacgggaagaacctggtgcaggaatggctggcaaagcaccagggtgcctggtatgtgtggaaccgcactgagctcatgcaggcgtccctggaccagtctgtgacccatctcatgggcctctttgagcccggagacacgaaatatgagatccaccgagaccccacactggacccctccctgatggagatgacagaggctgccctgcgcctgctgagcaggaacccccgcggcttctacctctttgtggagggcggccgcatcgaccatggtcatcatgagggtgtggcttaccaggcactcactgaggcggtcatgttcgacgacgccattgagagggcgggccagctcaccagcgaggaggacacgctgaccctcgtcaccgctgaccactcccatgtcttctcctttggtggctacaccttgcgagggagctccatcttcgggttggcccccagcaaggctcaggacagcaaagcctacacgtccatcctgtacggcaatggcccgggctacgtgttcaactcaggcgtgcgaccagacgtgaatgagagcgagagcgggagccccgattaccagcagcaggcggcggtgcccctgtcgtccgagacccacggaggcgaagacgtggcggtgtttgcgcgcggcccgcaggcgcacctggtgcatggtgtgcaggagcagagcttcgtagcgcatgtcatggccttcgctgcctgtctggagccctacacggcctgcgacctggcgcctcccgcctgcaccaccgacgccgcgcacccagttgccgcgtcgctgccactgctggccgggaccctgctgctgctgggggcgtccgctgctccctgatttactaaaaccttgaaataaaattgtaaaacatcagtttgaaggcctgactctcagggtagttcttttttaattctgggtttt

SEQ ID NO: 14 - DNA, 1672 bp, Artificial Sequence
  Synthetic polymer
atgcagtgggcctgtgtgctgctgctgctgggcctgtggctacagctctccctcaccttcatcccaggtaatcaggcggctcccagcagcccctactcacaggggcggctctaggctgacctgaccaacactctccccttgggcagctgaggaggaagaccccgccttctggaaccgccaggcagcccaggcccttgatgtagccaagaagttgcagccgatccagacagctgccaagaatgtcatcctcttcttgggggatgggatgggggtgcctacggtgacagccactcggatcctaaaggggcagatgaatggtaagctgggacctgagacacccctggccatggaccagttcccatacgtggctctgtccaagacatacaacgtggacagacaggtgccagacagcgcaggcactgccactgcctacctgtgtggggtcaagggcaactacaaaaccattggtgtaagtgcagccgcccgctacaaccagtgcaacacaacaagtggcaatgaggtcacgtctgtgatgaaccgggccaagaaagcaggaaagtcagtgggagtggtgaccacctccagggtgcagcatgcctccccagccggtgcttatgcacacacggtgaaccgaaactggtactcagatgccgacctgcctgccgatgcacagacgtatggctgccaggacatcgccacacaactggtcaacaacatggatattgacgtgatcctgggtggaggccgaatgtacatgtttcctgaggggaccccggatcctgaatacccatacgatgtcaatcagactggagtccggaaggacaagcggaatctggtgcaggagtggcaggccaagcaccagggagcccagtatgtgtggaaccgcacggagctccttcaggcagccaatgaccccagtgtaacacacctcatgggcctctttgagccggcagacatgaagtataatgttcagcaagaccccaccaaggacccgaccctggaggagatgacggaggcggccctgcaagtgctgagcaggaacccccagggcttctacctcttcgtggagggaggccgcattgaccacggtcaccatgaaggcaaagcttatatggcactgactgatacagtcatgtttgacaatgccatcgccaaggctaacgagctcactagcgaactggacacgctgatccttgccactgcagaccactcccatgtcttctcttttggtggctacacactgcgtgggacctccattttcggtctggcccccagcaaggcctcagacaacaagtcctacacctccatcctctatggcaatggccctggctacgtgcttggtgggggcttaaggcccgatgttaatgacagcataagcgaggacccctcgtaccggcagcaggcggccgtgcccctgtctagtgagtcccacgggggcgaggacgtggcggtgttcgcgcgaggcccgcaggcgcacctggtgcacggcgtgcaggaggagaccttcgtggcgcacgtcatggcctttgcgggctgcgtggagccctacaccgactgcaatctgccggccccctctggcctctccgacgccgcgcacctggcggccagcccgccttcgctggcgctgctggccggggcgatgctgctgctgctggcgcctgccttgtactga

SEQ ID NO: 15 - DNA, 1869 bp, Artificial Sequence
  Synthetic polymer
atgcagtgggcctgtgtgctgctgctgctgggcctgtggctacagctctccctcaccttcatcccagctgaggaggaagaccccgccttctggaaccgccaggcagcccaggcccttgatgtagccaagaagttgcagccgatccagacagctgccaagaatgtcatcctcttcttgggggatgggatgggggtgcctacggtgacagccactcggatcctaaaggggcagatgaatggtaagctgggacctgagacacccctggccatggaccagttcccatacgtggctctgtccaagacatacaacgtggacagacaggtgccagacagcgcaggcactgccactgcctacctgtgtggggtcaagggcaactacaaaaccattggtgtaagtgcagccgcccgctacaaccagtgcaacacaacaagtggcaatgaggtcacgtctgtgatgaaccgggccaagaaagcaggaaagtcagtgggagtggtgaccacctccagggtgcagcatgcctccccagccggtgcttatgcacacacggtgaaccgaaactggtactcagatgccgacctgcctgccgatgcacagacgtatggctgccaggacatcgccacacaactggtcaacaacatggatattgacgtgatcctgggtggaggccgaatgtacatgtttcctgaggggaccccggatcctgaatacccatacgatgtcaatcagactggagtccggaaggacaagcggaatctggtgcaggagtggcaggccaagcaccagggagcccagtatgtgtggaaccgcacggagctccttcaggcagccaatgaccccagtgtaacacacctcatgggcctctttgagccggcagacatgaagtataatgttcagcaagaccccaccaaggacccgaccctggaggagatgacggaggcggccctgcaagtgctgagcaggaacccccagggcttctacctcttcgtggagggaggccgcattgaccacggtcaccatgaaggcaaagcttatatggcactgactgatacagtcatgtttgacaatgccatcgccaaggctaacgagctcactagcgaactggacacgctgatccttgccactgcagaccactcccatgtcttctcttttggtggctacacactgcgtgggacctccattttcggtctggcccccagcaaggcctcagacaacaagtcctacacctccatcctctatggcaatggccctggctacgtgcttggtgggggcttaaggcccgatgttaatgacagcataagcgaggacccctcgtaccggcagcaggcggccgtgcccctgtctagtgagtcccacgggggcgaggacgtggcggtgttcgcgcgaggcccgcaggcgcacctggtgcacggcgtgcaggaggagaccttcgtggcgcacgtcatggcctttgcgggctgcgtggagccctacaccgactgcaatctgccggccccctctggcctctccgacgccgcgcacctggcggccagcccgccttcgctggcgctgctggccggggcgatgctgctgctgctggcgcctgccttgtactgaggggacccgggggtggggacacaggccccgccctccctgggaggcaggaagcagctctcaaataaactgttctaagtatgatacaggagtgatacatgtgtgaagagaagcccttaggtgggggcacagagtgtctgggtgaggggggtcagggtcacatcaggaggttagggaggggttgatgaagggctgacgttgagcaaagaccaaaggcaactcagaaggacagtggtgcaggactgggtgtggtcagcagggggactggttgggggatcc

SEQ ID NO: 16 - DNA, 1260 bp, Artificial Sequence
  Synthetic polymer
aaaaaacaagacaaagctgagatcagaaatgtcattgtgatgataggcgacggcatggggacgccttacataagagcctaccgttccatgaaaaataacggtgacacaccgaataacccgaagttaacagaatttgaccggaacctgacaggcatgatgatgacgcatccggatgaccctgactataatattacagattcagcagcagccggaacagcattagcgacaggcgttaagacatataacaatgcaattggcgtcgataaaaacggaaaaaaagtgaaatctgtacttgaagaggccaaacagcaaggcaagtcaacagggcttgtcgccacgtctgaaattaaccacgccactccagccgcatatggcgcccacaatgaatcacggaaaaacatggaccaaatcgccaacagctatatggatgacaagataaaaggcaaacataaaatagacgtgctgctcggcggcggaaaatcttattttaaccgcaagaacagaaacttgacaaaggaattcaaacaagccggctacagctatgtgacaactaaacaagcattgaaaaaaaataaagatcagcaggtgctcgggcttttcgcagatggagggcttgctaaagcgctcgaccgtgacagtaaaacaccgtctctcaaagacatgacggtttcagcaattgatcgcctgaaccaaaataaaaaaggatttttcttgatggtcgaagggagccagattgactgggcggcccatgacaatgatacagtaggagccatgagcgaggttaaagattttgaacaggcctataaagccgcgattgaatttgcgaaaaaagacaaacatacacttgtgattgcaactgctgaccatacaaccggcggctttaccattggcgcaaacggggaaaagaattggcacgcagaaccgattctctccgctaagaaaacacctgaattcatggccaaaaaaatcagtgaaggcaagccggttaaagatgtgctcgcccgctatgccaatctgaaagtcacatctgaagaaatcaaaagcgttgaagcagctgcacaggctgacaaaagcaaaggggcctccaaagccatcatcaagatttttaatacccgctccaacagcggatggacgagtaccgatcataccggcgaagaagtaccggtatacgcgtacggccccggaaaagaaaaattccgcggattgattaacaatacggaccaggcaaacatcatatttaagattttaaaaactggaaaa

SEQ ID NO: 17 - protein, 420 aa, Artificial Sequence
  Synthetic polymer
KKQDKAEIRNVIVMIGDGMGTPYIRAYRSMKNNGDTPNNPKLTEFDRNLTGMMMTHPDDPDYNITDSAAAGTALATGVKTYNNAIGVDKNGKKVKSVLEEAKQQGKSTGLVATSEINHATPAAYGAHNESRKNMDQIANSYMDDKIKGKHKIDVLLGGGKSYFNRKNRNLTKEFKQAGYSYVTTKQALKKNKDQQVLGLFADGGLAKALDRDSKTPSLKDMTVSAIDRLNQNKKGFFLMVEGSQIDWAAHDNDTVGAMSEVKDFEQAYKAAIEFAKKDKHTLVIATADHTTGGFTIGANGEKNWHAEPILSAKKTPEFMAKKISEGKPVKDVLARYANLKVTSEEIKSVEAAAQADKSKGASKAIIKIFNTRSNSGWTSTDHTGEEVPVYAYGPGKEKFRGLINNTDQANIIFKILKTGK

SEQ ID NO: 18 - protein, 776 aa, Artificial Sequence
  Synthetic polymer
MQGPWVLLLLGLRLQLSLGVIPAEEENPAFWNRQAAEALDAAKKLQPIQKVAKNLILFLGDGLGVPTVTATRILKGQKNGKLGPETPLAMDRFPYLALSKTYNVDRQVPDSAATATAYLCGVKANFQTIGLSAAARFNQCNTTRGNEVISVMNRAKQAGKSVGVVTTTRVQHASPAGTYAHTVNRNWYSDADMPASARQEGCQDIATQLISNMDIDVILGGGRKYMFPMGTPDPEYPADASQNGIRLDGKNLVQEWLAKHQGAWYVWNRTELMQASLDQSVTHLMGLFEPGDTKYEIHRDPTLDPSLMEMTEAALRLLSRNPRGFYLFVEGGRIDHGHHEGVAYQALTEAVMFDDAIERAGQLTSEEDTLTLVTADHSHVFSFGGYTLRGSSIFGLAPSKAQDSKAYTSILYGNGPGYVFNSGVRPDVNESESGSPDYQQQAAVPLSSETHGGEDVAVFARGPQAHLVHGVQEQSFVAHVMAFAACLEPYTACDLAPPACTTDAAHPVAASLPLLAGTLLLLGASAAPGGSGGSGGGGSGGGGSEPKSCDKTHTCPPCPAPELLGGPSVFLFPPKPKDTLMISRTPEVTCVVVDVSHEDPQVKFNWYVDGVQVHNAKTKPREQQYNSTYRVVSVLTVLHQNWLDGKEYKCKVSNKALPAPIEKTISKAKGQPREPQVYTLPPSREEMTKNQVSLTCLVKGFYPSDIAVEWESNGQPENNYKTTPPVLDSDGSFFLYSKLTVDKSRWQQGNVFSCSVMHEALHNHYTQKSLSLSPGK

SEQ ID NO: 19 - DNA, 18 bp, Artificial Sequence
  Synthetic polymer
catggaccgcttcccata

SEQ ID NO: 20 - DNA, 20 bp, Artificial Sequence
  Synthetic polymer
cttgcactgtctggaacctg

SEQ ID NO: 21 - DNA, 20 bp, Artificial Sequence
  Synthetic polymer
cagcgatgcccacaggaaag

SEQ ID NO: 22 - DNA, 19 bp, Artificial Sequence
  Synthetic polymer
acggagcccttgacgagag

SEQ ID NO: 23 - DNA, 20 bp, Artificial Sequence
  Synthetic polymer
cgtttccggttcaagctcac

SEQ ID NO: 24 - DNA, 23 bp, Artificial Sequence
  Synthetic polymer
cctgatgactttgatgctgaacg

SEQ ID NO: 25 - DNA, 20 bp, Artificial Sequence
  Synthetic polymer
actccttctgtgactccagc

SEQ ID NO: 26 - DNA, 20 bp, Artificial Sequence
  Synthetic polymer
ataactgcacccacttccca

SEQ ID NO: 27 - DNA, 23 bp, Artificial Sequence
  Synthetic polymer
gcactacaggctccgagatgaac

SEQ ID NO: 28 - DNA, 24 bp, Artificial Sequence
  Synthetic polymer
ttgtcgttgcttggttctccttgt

SEQ ID NO: 29 - DNA, 21 bp, Artificial Sequence
  Synthetic polymer
cctctggtcttctggagtacc

SEQ ID NO: 30 - DNA, 20 bp, Artificial Sequence
  Synthetic polymer
actccttctgtgactccagc

SEQ ID NO: 31 - DNA, 20 bp, Artificial Sequence
  Synthetic polymer
tctccaccgcaatgaagacc

SEQ ID NO: 32 - DNA, 20 bp, Artificial Sequence
  Synthetic polymer
cacacccaccagcatcttct

SEQ ID NO: 33 - DNA, 20 bp, Artificial Sequence
  Synthetic polymer
gctaagagcacagcaatgga

SEQ ID NO: 34 - DNA, 20 bp, Artificial Sequence
  Synthetic polymer
gcatgttcaacgttatccat

SEQ ID NO: 35 - DNA, 19 bp, Artificial Sequence
  Synthetic polymer
cacgcaatcctggatgtca

SEQ ID NO: 36 - DNA, 18 bp, Artificial Sequence
  Synthetic polymer
gtcgcgcctgctgttgct

SEQ ID NO: 37 - DNA, 23 bp, Artificial Sequence
  Synthetic polymer
ccccatctgactatgtggaaaga

SEQ ID NO: 38 - DNA, 23 bp, Artificial Sequence
  Synthetic polymer
aaaaccgcttgtcattcactttg

SEQ ID NO: 39 - DNA, 23 bp, Artificial Sequence
  Synthetic polymer
caggagcgagaccccactaacat

SEQ ID NO: 40 - DNA, 23 bp, Artificial Sequence
  Synthetic polymer
gtcagatccacgacggacacatt

SEQ ID NO: 41 - protein, 16 aa, Artificial Sequence
  Synthetic polymer
GGSGGSGGGGSGGGGS

SEQ ID NO: 42 - protein, 5 aa, Artificial Sequence
  Synthetic polymer
GGGGS

SEQ ID NO: 43 - protein, 10 aa, Artificial Sequence
  Synthetic polymer
GGGGSGGGGS

SEQ ID NO: 44 - protein, 15 aa, Artificial Sequence
  Synthetic polymer
GGGGSGGGGSGGGGS

SEQ ID NO: 45 - protein, 20 aa, Artificial Sequence
  Synthetic polymer
GGGGSGGGGSGGGGSGGGGS

SEQ ID NO: 46 - protein, 8 aa, Artificial Sequence
  Synthetic polymer
GGGGGGGG

SEQ ID NO: 47 - protein, 6 aa, Artificial Sequence
  Synthetic polymer
GGGGGG

SEQ ID NO: 48 - protein, 5 aa, Artificial Sequence
  Synthetic polymer
EAAAK

SEQ ID NO: 49 - protein, 10 aa, Artificial Sequence
  Synthetic polymer
EAAAKEAAAK

SEQ ID NO: 50 - protein, 15 aa, Artificial Sequence
  Synthetic polymer
EAAAKEAAAKEAAAK

SEQ ID NO: 51 - protein, 12 aa, Artificial Sequence
  Synthetic polymer
AEAAAKEAAAKA

SEQ ID NO: 52 - protein, 17 aa, Artificial Sequence
  Synthetic polymer
AEAAAKEAAAKEAAAKA

SEQ ID NO: 53 - protein, 21 aa, Artificial Sequence
  Synthetic polymer
AEAAAKEAAAKEAAAKEAAAK

SEQ ID NO: 54 - protein, 27 aa, Artificial Sequence
  Synthetic polymer
AEAAAKEAAAKEAAAKEAAAKEAAAKA

SEQ ID NO: 55 - protein, 12 aa, Artificial Sequence
  Synthetic polymer
AEAAAKEAAAKA

SEQ ID NO: 56 - protein, 46 aa, Artificial Sequence
  Synthetic polymer
AEAAAKEAAAKEAAAKEAAAKALEAEAAAKEAAAKEAAAKEAAAKA

SEQ ID NO: 57 - protein, 5 aa, Artificial Sequence
  Synthetic polymer
PAPAP

SEQ ID NO: 58 - protein, 18 aa, Artificial Sequence
  Synthetic polymer
KESGSVSSEQLAQFRSLD

SEQ ID NO: 59 - protein, 14 aa, Artificial Sequence
  Synthetic polymer
EGKSSGSGSESKST

SEQ ID NO: 60 - protein, 12 aa, Artificial Sequence
  Synthetic polymer
GSAGSAAGSGEF